European Patent Specification EP 4 095 263 B1, published July 8, 2026. Title: METHODS OF ASSESSING NUCLEASE CLEAVAGE. Applicant: EDITAS MEDICINE, INC. Application PCT/US2018/012652. The sequence listing filed with the application follows.

SEQUENCE LISTING (94 sequences)

SEQ ID NO: 1 - DNA, 65 bp, Artificial Sequence
  source: /note="Description of Artificial Sequence: Synthetic primer"
caccgctagctaatacgactcactataggccacggagcgagacatctgttttagagctagaaata

SEQ ID NO: 2 - DNA, 65 bp, Artificial Sequence
  source: /note="Description of Artificial Sequence: Synthetic primer"
caccgctagctaatacgactcactatagctggtacacggcagggtcagttttagagctagaaata

SEQ ID NO: 3 - DNA, 53 bp, Artificial Sequence
  source: /note="Description of Artificial Sequence: Synthetic primer"
ttttttttttttttttttttgcaccgactcggtgccactttttcaagttgata

SEQ ID NO: 4 - DNA, 64 bp, Artificial Sequence
  source: /note="Description of Artificial Sequence: Synthetic primer"
gtgactggagttcagacgtgtgctcttccgatctggaccatggatgcactctgtaaattctcat

SEQ ID NO: 5 - DNA, 65 bp, Artificial Sequence
  source: /note="Description of Artificial Sequence: Synthetic primer"
gtgactggagttcagacgtgtgctcttccgatctgcatgccttcttaaacatcacgagactctaa

SEQ ID NO: 6 - DNA, 64 bp, Artificial Sequence
  source: /note="Description of Artificial Sequence: Synthetic primer"
gtgactggagttcagacgtgtgctcttccgatctgcactgttgctcttgaagtccatagacctc

SEQ ID NO: 7 - DNA, 80 bp, Artificial Sequence
  source: /note="Description of Artificial Sequence: Synthetic oligonucleotide"
  modified_base (38)..(47): a, c, t, g, unknown or other
aatgatacggcgaccaccgagatctacactagatcgcnnnnnnnnnntcgtcggcagcgtcagatgtgtataagagacag

SEQ ID NO: 8 - DNA, 80 bp, Artificial Sequence
  source: /note="Description of Artificial Sequence: Synthetic oligonucleotide"
  modified_base (38)..(47): a, c, t, g, unknown or other
aatgatacggcgaccaccgagatctacacctctctatnnnnnnnnnntcgtcggcagcgtcagatgtgtataagagacag

SEQ ID NO: 9 - DNA, 80 bp, Artificial Sequence
  source: /note="Description of Artificial Sequence: Synthetic oligonucleotide"
  modified_base (38)..(47): a, c, t, g, unknown or other
aatgatacggcgaccaccgagatctacactatcctctnnnnnnnnnntcgtcggcagcgtcagatgtgtataagagacag

SEQ ID NO: 10 - DNA, 80 bp, Artificial Sequence
  source: /note="Description of Artificial Sequence: Synthetic oligonucleotide"
  modified_base (38)..(47): a, c, t, g, unknown or other
aatgatacggcgaccaccgagatctacacagagtagannnnnnnnnntcgtcggcagcgtcagatgtgtataagagacag

SEQ ID NO: 11 - DNA, 80 bp, Artificial Sequence
  source: /note="Description of Artificial Sequence: Synthetic oligonucleotide"
  modified_base (38)..(47): a, c, t, g, unknown or other
aatgatacggcgaccaccgagatctacacgtaaggagnnnnnnnnnntcgtcggcagcgtcagatgtgtataagagacag

SEQ ID NO: 12 - DNA, 80 bp, Artificial Sequence
  source: /note="Description of Artificial Sequence: Synthetic oligonucleotide"
  modified_base (38)..(47): a, c, t, g, unknown or other
aatgatacggcgaccaccgagatctacacactgcatannnnnnnnnntcgtcggcagcgtcagatgtgtataagagacag

SEQ ID NO: 13 - DNA, 80 bp, Artificial Sequence
  source: /note="Description of Artificial Sequence: Synthetic oligonucleotide"
  modified_base (38)..(47): a, c, t, g, unknown or other
aatgatacggcgaccaccgagatctacacaaggagtannnnnnnnnntcgtcggcagcgtcagatgtgtataagagacag

SEQ ID NO: 14 - DNA, 80 bp, Artificial Sequence
  source: /note="Description of Artificial Sequence: Synthetic oligonucleotide"
  modified_base (38)..(47): a, c, t, g, unknown or other
aatgatacggcgaccaccgagatctacacctaagcctnnnnnnnnnntcgtcggcagcgtcagatgtgtataagagacag

SEQ ID NO: 15 - DNA, 15 bp, Artificial Sequence
  source: /note="Description of Artificial Sequence: Synthetic oligonucleotide"
ctgtctcttatacac

SEQ ID NO: 16 - DNA, 29 bp, Artificial Sequence
  source: /note="Description of Artificial Sequence: Synthetic primer"
aatgatacggcgaccaccgagatctacac

SEQ ID NO: 17 - DNA, 53 bp, Artificial Sequence
  source: /note="Description of Artificial Sequence: Synthetic primer"
caagcagaagacggcatacgagatagcggaatgtgactggagttcagacgtgt

SEQ ID NO: 18 - DNA, 53 bp, Artificial Sequence
  source: /note="Description of Artificial Sequence: Synthetic primer"
caagcagaagacggcatacgagatgatcatgcgtgactggagttcagacgtgt

SEQ ID NO: 19 - DNA, 53 bp, Artificial Sequence
  source: /note="Description of Artificial Sequence: Synthetic primer"
caagcagaagacggcatacgagataagacggagtgactggagttcagacgtgt

SEQ ID NO: 20 - DNA, 53 bp, Artificial Sequence
  source: /note="Description of Artificial Sequence: Synthetic primer"
caagcagaagacggcatacgagatcgagtcctgtgactggagttcagacgtgt

SEQ ID NO: 21 - DNA, 53 bp, Artificial Sequence
  source: /note="Description of Artificial Sequence: Synthetic primer"
caagcagaagacggcatacgagattcctcagggtgactggagttcagacgtgt

SEQ ID NO: 22 - DNA, 53 bp, Artificial Sequence
  source: /note="Description of Artificial Sequence: Synthetic primer"
caagcagaagacggcatacgagatgtacggatgtgactggagttcagacgtgt

SEQ ID NO: 23 - DNA, 53 bp, Artificial Sequence
  source: /note="Description of Artificial Sequence: Synthetic primer"
caagcagaagacggcatacgagatcatctctcgtgactggagttcagacgtgt

SEQ ID NO: 24 - DNA, 53 bp, Artificial Sequence
  source: /note="Description of Artificial Sequence: Synthetic primer"
caagcagaagacggcatacgagatgtcggagcgtgactggagttcagacgtgt

SEQ ID NO: 25 - DNA, 53 bp, Artificial Sequence
  source: /note="Description of Artificial Sequence: Synthetic primer"
caagcagaagacggcatacgagatacggagaagtgactggagttcagacgtgt

SEQ ID NO: 26 - DNA, 53 bp, Artificial Sequence
  source: /note="Description of Artificial Sequence: Synthetic primer"
caagcagaagacggcatacgagataggagatggtgactggagttcagacgtgt

SEQ ID NO: 27 - DNA, 53 bp, Artificial Sequence
  source: /note="Description of Artificial Sequence: Synthetic primer"
caagcagaagacggcatacgagatagtactcggtgactggagttcagacgtgt

SEQ ID NO: 28 - DNA, 53 bp, Artificial Sequence
  source: /note="Description of Artificial Sequence: Synthetic primer"
caagcagaagacggcatacgagatggactctagtgactggagttcagacgtgt

SEQ ID NO: 29 - DNA, 78 bp, Artificial Sequence
  source: /note="Description of Artificial Sequence: Synthetic oligonucleotide"
  modified_base (38)..(39): a, c, t, g, unknown or other
  modified_base (41)..(42): a, c, t, g, unknown or other
  modified_base (44)..(45): a, c, t, g, unknown or other
aatgatacggcgaccaccgagatctacacactgcatannwnnwnnacactctttccctacacgacgctcttccgatct

SEQ ID NO: 30 - DNA, 78 bp, Artificial Sequence
  source: /note="Description of Artificial Sequence: Synthetic oligonucleotide"
  modified_base (38)..(39): a, c, t, g, unknown or other
  modified_base (41)..(42): a, c, t, g, unknown or other
  modified_base (44)..(45): a, c, t, g, unknown or other
aatgatacggcgaccaccgagatctacacaaggagtannwnnwnnacactctttccctacacgacgctcttccgatct

SEQ ID NO: 31 - DNA, 14 bp, Artificial Sequence
  source: /note="Description of Artificial Sequence: Synthetic oligonucleotide"
gatcggaagagcca

SEQ ID NO: 32 - DNA, 15 bp, Artificial Sequence
  source: /note="Description of Artificial Sequence: Synthetic oligonucleotide"
ctgtctcttatacac

SEQ ID NO: 33 - DNA, 80 bp, Artificial Sequence; identical to SEQ ID NO: 7
  source: /note="Description of Artificial Sequence: Synthetic oligonucleotide"
  modified_base (38)..(47): a, c, t, g, unknown or other

SEQ ID NO: 34 - DNA, 80 bp, Artificial Sequence; identical to SEQ ID NO: 8
  source: /note="Description of Artificial Sequence: Synthetic oligonucleotide"
  modified_base (38)..(47): a, c, t, g, unknown or other

SEQ ID NO: 35 - DNA, 80 bp, Artificial Sequence; identical to SEQ ID NO: 9
  source: /note="Description of Artificial Sequence: Synthetic oligonucleotide"
  modified_base (38)..(47): a, c, t, g, unknown or other

SEQ ID NO: 36 - DNA, 80 bp, Artificial Sequence; identical to SEQ ID NO: 10
  source: /note="Description of Artificial Sequence: Synthetic oligonucleotide"
  modified_base (38)..(47): a, c, t, g, unknown or other

SEQ ID NO: 37 - DNA, 80 bp, Artificial Sequence; identical to SEQ ID NO: 11
  source: /note="Description of Artificial Sequence: Synthetic oligonucleotide"
  modified_base (38)..(47): a, c, t, g, unknown or other

SEQ ID NO: 38 - DNA, 80 bp, Artificial Sequence; identical to SEQ ID NO: 12
  source: /note="Description of Artificial Sequence: Synthetic oligonucleotide"
  modified_base (38)..(47): a, c, t, g, unknown or other

SEQ ID NO: 39 - DNA, 80 bp, Artificial Sequence; identical to SEQ ID NO: 13
  source: /note="Description of Artificial Sequence: Synthetic oligonucleotide"
  modified_base (38)..(47): a, c, t, g, unknown or other

SEQ ID NO: 40 - DNA, 80 bp, Artificial Sequence; identical to SEQ ID NO: 14
  source: /note="Description of Artificial Sequence: Synthetic oligonucleotide"
  modified_base (38)..(47): a, c, t, g, unknown or other

SEQ ID NO: 41 - DNA, 18 bp, Artificial Sequence
  source: /note="Description of Artificial Sequence: Synthetic oligonucleotide"
tagatcgctttttttttt

SEQ ID NO: 42 - DNA, 18 bp, Artificial Sequence
  source: /note="Description of Artificial Sequence: Synthetic oligonucleotide"
ctctctattttttttttt

SEQ ID NO: 43 - DNA, 18 bp, Artificial Sequence
  source: /note="Description of Artificial Sequence: Synthetic oligonucleotide"
tatcctcttttttttttt

SEQ ID NO: 44 - DNA, 18 bp, Artificial Sequence
  source: /note="Description of Artificial Sequence: Synthetic oligonucleotide"
agagtagatttttttttt

SEQ ID NO: 45 - DNA, 18 bp, Artificial Sequence
  source: /note="Description of Artificial Sequence: Synthetic oligonucleotide"
gtaaggagtttttttttt

SEQ ID NO: 46 - DNA, 18 bp, Artificial Sequence
  source: /note="Description of Artificial Sequence: Synthetic oligonucleotide"
actgcatatttttttttt

SEQ ID NO: 47 - DNA, 18 bp, Artificial Sequence
  source: /note="Description of Artificial Sequence: Synthetic oligonucleotide"
aaggagtatttttttttt

SEQ ID NO: 48 - DNA, 18 bp, Artificial Sequence
  source: /note="Description of Artificial Sequence: Synthetic oligonucleotide"
ctaagccttttttttttt

SEQ ID NO: 49 - DNA, 29 bp, Artificial Sequence
  source: /note="Description of Artificial Sequence: Synthetic oligonucleotide"
aatgatacggcgaccaccgagatctacac

SEQ ID NO: 50 - DNA, 53 bp, Artificial Sequence; identical to SEQ ID NO: 17
  source: /note="Description of Artificial Sequence: Synthetic oligonucleotide"

SEQ ID NO: 51 - DNA, 53 bp, Artificial Sequence; identical to SEQ ID NO: 18
  source: /note="Description of Artificial Sequence: Synthetic oligonucleotide"

SEQ ID NO: 52 - DNA, 53 bp, Artificial Sequence; identical to SEQ ID NO: 19
  source: /note="Description of Artificial Sequence: Synthetic oligonucleotide"

SEQ ID NO: 53 - DNA, 53 bp, Artificial Sequence; identical to SEQ ID NO: 20
  source: /note="Description of Artificial Sequence: Synthetic oligonucleotide"

SEQ ID NO: 54 - DNA, 53 bp, Artificial Sequence; identical to SEQ ID NO: 21
  source: /note="Description of Artificial Sequence: Synthetic oligonucleotide"

SEQ ID NO: 55 - DNA, 53 bp, Artificial Sequence; identical to SEQ ID NO: 22
  source: /note="Description of Artificial Sequence: Synthetic oligonucleotide"

SEQ ID NO: 56 - DNA, 53 bp, Artificial Sequence; identical to SEQ ID NO: 23
  source: /note="Description of Artificial Sequence: Synthetic oligonucleotide"

SEQ ID NO: 57 - DNA, 53 bp, Artificial Sequence; identical to SEQ ID NO: 24
  source: /note="Description of Artificial Sequence: Synthetic oligonucleotide"

SEQ ID NO: 58 - DNA, 53 bp, Artificial Sequence; identical to SEQ ID NO: 25
  source: /note="Description of Artificial Sequence: Synthetic oligonucleotide"

SEQ ID NO: 59 - DNA, 53 bp, Artificial Sequence; identical to SEQ ID NO: 26
  source: /note="Description of Artificial Sequence: Synthetic oligonucleotide"

SEQ ID NO: 60 - DNA, 53 bp, Artificial Sequence; identical to SEQ ID NO: 27
  source: /note="Description of Artificial Sequence: Synthetic oligonucleotide"

SEQ ID NO: 61 - DNA, 53 bp, Artificial Sequence; identical to SEQ ID NO: 28
  source: /note="Description of Artificial Sequence: Synthetic oligonucleotide"

SEQ ID NO: 62 - DNA, 8 bp, Artificial Sequence
  source: /note="Description of Artificial Sequence: Synthetic oligonucleotide"
agcggaat

SEQ ID NO: 63 - DNA, 8 bp, Artificial Sequence
  source: /note="Description of Artificial Sequence: Synthetic oligonucleotide"
gatcatgc

SEQ ID NO: 64 - DNA, 8 bp, Artificial Sequence
  source: /note="Description of Artificial Sequence: Synthetic oligonucleotide"
aagacgga

SEQ ID NO: 65 - DNA, 8 bp, Artificial Sequence
  source: /note="Description of Artificial Sequence: Synthetic oligonucleotide"
cgagtcct

SEQ ID NO: 66 - DNA, 8 bp, Artificial Sequence
  source: /note="Description of Artificial Sequence: Synthetic oligonucleotide"
tcctcagg

SEQ ID NO: 67 - DNA, 8 bp, Artificial Sequence
  source: /note="Description of Artificial Sequence: Synthetic oligonucleotide"
gtacggat

SEQ ID NO: 68 - DNA, 8 bp, Artificial Sequence
  source: /note="Description of Artificial Sequence: Synthetic oligonucleotide"
catctctc

SEQ ID NO: 69 - DNA, 8 bp, Artificial Sequence
  source: /note="Description of Artificial Sequence: Synthetic oligonucleotide"
gtcggagc

SEQ ID NO: 70 - DNA, 8 bp, Artificial Sequence
  source: /note="Description of Artificial Sequence: Synthetic oligonucleotide"
acggagaa

SEQ ID NO: 71 - DNA, 8 bp, Artificial Sequence
  source: /note="Description of Artificial Sequence: Synthetic oligonucleotide"
aggagatg

SEQ ID NO: 72 - DNA, 8 bp, Artificial Sequence
  source: /note="Description of Artificial Sequence: Synthetic oligonucleotide"
agtactcg

SEQ ID NO: 73 - DNA, 8 bp, Artificial Sequence
  source: /note="Description of Artificial Sequence: Synthetic oligonucleotide"
ggactcta

SEQ ID NO: 74 - DNA, 8 bp, Artificial Sequence
  source: /note="Description of Artificial Sequence: Synthetic oligonucleotide"
attccgct

SEQ ID NO: 75 - DNA, 8 bp, Artificial Sequence
  source: /note="Description of Artificial Sequence: Synthetic oligonucleotide"
gcatgatg

SEQ ID NO: 76 - DNA, 8 bp, Artificial Sequence
  source: /note="Description of Artificial Sequence: Synthetic oligonucleotide"
tccgtctt

SEQ ID NO: 77 - DNA, 8 bp, Artificial Sequence
  source: /note="Description of Artificial Sequence: Synthetic oligonucleotide"
aggactcg

SEQ ID NO: 78 - DNA, 8 bp, Artificial Sequence
  source: /note="Description of Artificial Sequence: Synthetic oligonucleotide"
cctgagga

SEQ ID NO: 79 - DNA, 8 bp, Artificial Sequence
  source: /note="Description of Artificial Sequence: Synthetic oligonucleotide"
atccgtac

SEQ ID NO: 80 - DNA, 8 bp, Artificial Sequence
  source: /note="Description of Artificial Sequence: Synthetic oligonucleotide"
gagagatg

SEQ ID NO: 81 - DNA, 8 bp, Artificial Sequence
  source: /note="Description of Artificial Sequence: Synthetic oligonucleotide"
gctccgac

SEQ ID NO: 82 - DNA, 8 bp, Artificial Sequence
  source: /note="Description of Artificial Sequence: Synthetic oligonucleotide"
ttctccgt

SEQ ID NO: 83 - DNA, 8 bp, Artificial Sequence
  source: /note="Description of Artificial Sequence: Synthetic oligonucleotide"
catctcct

SEQ ID NO: 84 - DNA, 8 bp, Artificial Sequence
  source: /note="Description of Artificial Sequence: Synthetic oligonucleotide"
cgagtact

SEQ ID NO: 85 - DNA, 8 bp, Artificial Sequence
  source: /note="Description of Artificial Sequence: Synthetic oligonucleotide"
tagagtcc

SEQ ID NO: 86 - DNA, 37 bp, Artificial Sequence
  source: /note="Description of Artificial Sequence: Synthetic primer"
ccttagaaaccactgctaactgaaagagactaagatt

SEQ ID NO: 87 - DNA, 37 bp, Artificial Sequence
  source: /note="Description of Artificial Sequence: Synthetic primer"
atttggaaaccaatgcttactaaatgagactaagacg

SEQ ID NO: 88 - DNA, 71 bp, Artificial Sequence
  source: /note="Description of Artificial Sequence: Synthetic oligonucleotide"
gtgactggagttcagacgtgtgctcttccgatctccttagaaaccactgctaactgaaagagactaagatt

SEQ ID NO: 89 - DNA, 71 bp, Artificial Sequence
  source: /note="Description of Artificial Sequence: Synthetic oligonucleotide"
gtgactggagttcagacgtgtgctcttccgatctatttggaaaccaatgcttactaaatgagactaagacg

SEQ ID NO: 90 - DNA, 10 bp, Artificial Sequence
  source: /note="Description of Artificial Sequence: Synthetic oligonucleotide"
tttttttttt

SEQ ID NO: 91 - DNA, 184 bp, Artificial Sequence
  source: /note="Description of Artificial Sequence: Synthetic polynucleotide"
  modified_base (6)..(7): a, c, t, g, unknown or other
  modified_base (9)..(9): a, c, t, g, unknown or other
  modified_base (46)..(46): a, c, t, g, unknown or other
tagranntnttttcactrcactawtgagaamttaagagataatggncwaaarycacaragagtatattcaaarakaagtatagcacttyttmyttrgaaaccamtgctwactraawgagactaagayktgtcccrtcaaaaatcctggacctatgcctaaaacacatttcacaatccctgaact

SEQ ID NO: 92 - DNA, 183 bp, Unknown
  source: /note="Description of Unknown: HGB1 sequence"
tagaaattgttttcactgcactattgagaaattaagagataatggcaaaagtcacaaagagtatattcaaaaagaagtatagcactttttccttagaaaccactgctaactgaaagagactaagatttgtcccgtcaaaaatcctggacctatgcctaaaacacatttcacaatccctgaact

SEQ ID NO: 93 - DNA, 181 bp, Unknown
  source: /note="Description of Unknown: HBG2 sequence"
taggatttttcactacactaatgagaacttaagagataatggcctaaaaccacagagagtatattcaaagataagtatagcacttcttatttggaaaccaatgcttactaaatgagactaagacgtgtcccatcaaaaatcctggacctatgcctaaaacacatttcacaatccctgaact

SEQ ID NO: 94 - DNA, 40 bp, Artificial Sequence
  source: /note="Description of Artificial Sequence: Synthetic oligonucleotide"
cagccacttgaactctatacgtatagagttcaagtggctg